European Patent Application EP 4 365 288 A1, published May 8, 2024. Title: Polynucleotide and pharmaceutical composition. Applicant: Kyowa Kirin Co., Ltd. National University Corporation Tokai National H. The sequence listing filed with the application follows.

SEQUENCE LISTING (480 sequences)

SEQ ID NO: 1 - RNA, 145 nt, Artificial Sequence
  E1
gggagaauacaagcuacuuguucuuuuugcagccaccauggacuacaaggacgacgacgacaagaucaucgacuauaaagacgacgacgauaaagguggcgacuauaaggacgacgacgacaaacaccaccaccaccaccacuga

SEQ ID NO: 2 - RNA, 80 nt, Artificial Sequence
  E1-1
gggagaauacaagcuacuuguucuuuuugcagccaccauggacuacaaggacgacgacgacaagaucaucgacuauaaag

SEQ ID NO: 3 - RNA, 80 nt, Artificial Sequence; identical to SEQ ID NO: 2
  E1-2

SEQ ID NO: 4 - DNA, 30 bp, Artificial Sequence
  template DNA 1
cctttatcgtcgtcgtctttatagtcgatg

SEQ ID NO: 5 - DNA, 165 bp, Artificial Sequence
  E2
gggagaauacaagcuacuuguucuuuuugcagccaccauggacuacaaggacgacgacgacaagaucaucgacuauaaagacgacgacgauaaagguggcgacuauaaggacgacgacgacaaacaccaccaccaccaccactgaaaaaaaaaaaaaaaaaaaaa

SEQ ID NO: 6 - RNA, 80 nt, Artificial Sequence; identical to SEQ ID NO: 2
  E2-1

SEQ ID NO: 7 - DNA, 85 bp, Artificial Sequence
  E2-2
acgacgacgauaaagguggcgacuauaaggacgacgacgacaaacaccaccaccaccaccactgaaaaaaaaaaaaaaaaaaaaa

SEQ ID NO: 8 - RNA, 145 nt, Artificial Sequence; identical to SEQ ID NO: 1
  E3

SEQ ID NO: 9 - RNA, 80 nt, Artificial Sequence; identical to SEQ ID NO: 2
  E3-1

SEQ ID NO: 10 - RNA, 65 nt, Artificial Sequence
  E3-2
acgacgacgauaaagguggcgacuauaaggacgacgacgacaaacaccaccaccaccaccacuga

SEQ ID NO: 11 - RNA, 165 nt, Artificial Sequence
  E4
gggagaauacaagcuacuuguucuuuuugcagccaccauggacuacaaggacgacgacgacaagaucaucgacuauaaagacgacgacgauaaagguggcgacuauaaggacgacgacgacaaacaccaccaccaccaccacugaaaaaaaaaaaaaaaaaaaaa

SEQ ID NO: 12 - RNA, 80 nt, Artificial Sequence; identical to SEQ ID NO: 2
  E4-1

SEQ ID NO: 13 - RNA, 85 nt, Artificial Sequence
  E4-2
acgacgacgauaaagguggcgacuauaaggacgacgacgacaaacaccaccaccaccaccacugaaaaaaaaaaaaaaaaaaaaa

SEQ ID NO: 14 - RNA, 145 nt, Artificial Sequence; identical to SEQ ID NO: 1
  E5

SEQ ID NO: 15 - RNA, 80 nt, Artificial Sequence; identical to SEQ ID NO: 2
  E5-1

SEQ ID NO: 16 - RNA, 65 nt, Artificial Sequence; identical to SEQ ID NO: 10
  E5-2

SEQ ID NO: 17 - RNA, 145 nt, Artificial Sequence; identical to SEQ ID NO: 1
  E6

SEQ ID NO: 18 - RNA, 80 nt, Artificial Sequence; identical to SEQ ID NO: 2
  E6-1

SEQ ID NO: 19 - RNA, 65 nt, Artificial Sequence; identical to SEQ ID NO: 10
  E6-2

SEQ ID NO: 20 - RNA, 165 nt, Artificial Sequence; identical to SEQ ID NO: 11
  E7

SEQ ID NO: 21 - RNA, 80 nt, Artificial Sequence; identical to SEQ ID NO: 2
  E7-1

SEQ ID NO: 22 - RNA, 85 nt, Artificial Sequence; identical to SEQ ID NO: 13
  E7-2

SEQ ID NO: 23 - RNA, 165 nt, Artificial Sequence; identical to SEQ ID NO: 11
  E8

SEQ ID NO: 24 - RNA, 80 nt, Artificial Sequence; identical to SEQ ID NO: 2
  E8-1

SEQ ID NO: 25 - RNA, 85 nt, Artificial Sequence; identical to SEQ ID NO: 13
  E8-2

SEQ ID NO: 26 - RNA, 165 nt, Artificial Sequence; identical to SEQ ID NO: 11
  E9

SEQ ID NO: 27 - RNA, 80 nt, Artificial Sequence; identical to SEQ ID NO: 2
  E9-1

SEQ ID NO: 28 - RNA, 85 nt, Artificial Sequence; identical to SEQ ID NO: 13
  E9-2

SEQ ID NO: 29 - RNA, 145 nt, Artificial Sequence; identical to SEQ ID NO: 1
  E10

SEQ ID NO: 30 - RNA, 80 nt, Artificial Sequence; identical to SEQ ID NO: 2
  E10-1

SEQ ID NO: 31 - RNA, 65 nt, Artificial Sequence; identical to SEQ ID NO: 10
  E10-2

SEQ ID NO: 32 - RNA, 165 nt, Artificial Sequence; identical to SEQ ID NO: 11
  E11

SEQ ID NO: 33 - RNA, 80 nt, Artificial Sequence; identical to SEQ ID NO: 2
  E11-1

SEQ ID NO: 34 - RNA, 85 nt, Artificial Sequence; identical to SEQ ID NO: 13
  E11-2

SEQ ID NO: 35 - RNA, 165 nt, Artificial Sequence; identical to SEQ ID NO: 11
  E12

SEQ ID NO: 36 - RNA, 80 nt, Artificial Sequence; identical to SEQ ID NO: 2
  E12-1

SEQ ID NO: 37 - RNA, 85 nt, Artificial Sequence; identical to SEQ ID NO: 13
  E12-2

SEQ ID NO: 38 - RNA, 165 nt, Artificial Sequence; identical to SEQ ID NO: 11
  E13

SEQ ID NO: 39 - RNA, 80 nt, Artificial Sequence; identical to SEQ ID NO: 2
  E13-1

SEQ ID NO: 40 - RNA, 85 nt, Artificial Sequence; identical to SEQ ID NO: 13
  E13-2

SEQ ID NO: 41 - RNA, 165 nt, Artificial Sequence; identical to SEQ ID NO: 11
  E14

SEQ ID NO: 42 - RNA, 80 nt, Artificial Sequence; identical to SEQ ID NO: 2
  E14-1

SEQ ID NO: 43 - RNA, 85 nt, Artificial Sequence; identical to SEQ ID NO: 13
  E14-2

SEQ ID NO: 44 - RNA, 165 nt, Artificial Sequence; identical to SEQ ID NO: 11
  E15

SEQ ID NO: 45 - RNA, 80 nt, Artificial Sequence; identical to SEQ ID NO: 2
  E15-1

SEQ ID NO: 46 - RNA, 85 nt, Artificial Sequence; identical to SEQ ID NO: 13
  E15-2

SEQ ID NO: 47 - RNA, 165 nt, Artificial Sequence; identical to SEQ ID NO: 11
  E16

SEQ ID NO: 48 - RNA, 80 nt, Artificial Sequence; identical to SEQ ID NO: 2
  E16-1

SEQ ID NO: 49 - RNA, 85 nt, Artificial Sequence; identical to SEQ ID NO: 13
  E16-2

SEQ ID NO: 50 - RNA, 165 nt, Artificial Sequence; identical to SEQ ID NO: 11
  E17

SEQ ID NO: 51 - RNA, 80 nt, Artificial Sequence; identical to SEQ ID NO: 2
  E17-1

SEQ ID NO: 52 - RNA, 85 nt, Artificial Sequence; identical to SEQ ID NO: 13
  E17-2

SEQ ID NO: 53 - RNA, 145 nt, Artificial Sequence; identical to SEQ ID NO: 1
  E18

SEQ ID NO: 54 - RNA, 80 nt, Artificial Sequence; identical to SEQ ID NO: 2
  E18-1

SEQ ID NO: 55 - RNA, 65 nt, Artificial Sequence; identical to SEQ ID NO: 10
  E18-2

SEQ ID NO: 56 - RNA, 145 nt, Artificial Sequence
  E19
  misc_feature (4)..(4): Am6(M)
  misc_feature (6)..(7): Am6(M)
  misc_feature (9)..(9): Am6(M)
  misc_feature (11)..(12): Am6(M)
  misc_feature (16)..(16): Am6(M)
  misc_feature (31)..(31): Am6(M)
gggngnnuncnngcuncuuguucuuuuugcngccaccauggacuacaaggacgacgacgacaagaucaucgacuauaaagacgacgacgauaaagguggcgacuauaaggacgacgacgacaaacaccaccaccaccaccacuga

SEQ ID NO: 57 - RNA, 80 nt, Artificial Sequence
  E19-1
  misc_feature (4)..(4): Am6(M)
  misc_feature (6)..(7): Am6(M)
  misc_feature (9)..(9): Am6(M)
  misc_feature (11)..(12): Am6(M)
  misc_feature (16)..(16): Am6(M)
  misc_feature (31)..(31): Am6(M)
gggngnnuncnngcuncuuguucuuuuugcngccaccauggacuacaaggacgacgacgacaagaucaucgacuauaaag

SEQ ID NO: 58 - RNA, 65 nt, Artificial Sequence; identical to SEQ ID NO: 10
  E19-2

SEQ ID NO: 59 - RNA, 145 nt, Artificial Sequence; identical to SEQ ID NO: 56
  E20
  misc_feature (4)..(4): Am6(F)
  misc_feature (6)..(7): Am6(F)
  misc_feature (9)..(9): Am6(F)
  misc_feature (11)..(12): Am6(F)
  misc_feature (16)..(16): Am6(F)
  misc_feature (31)..(31): Am6(F)

SEQ ID NO: 60 - RNA, 80 nt, Artificial Sequence; identical to SEQ ID NO: 57
  E20-1
  misc_feature (4)..(4): Am6(F)
  misc_feature (6)..(7): Am6(F)
  misc_feature (9)..(9): Am6(F)
  misc_feature (11)..(12): Am6(F)
  misc_feature (16)..(16): Am6(F)
  misc_feature (31)..(31): Am6(F)

SEQ ID NO: 61 - RNA, 65 nt, Artificial Sequence; identical to SEQ ID NO: 10
  E20-2

SEQ ID NO: 62 - RNA, 145 nt, Artificial Sequence
  E21
  misc_feature (4)..(4): Am6(F)
  misc_feature (6)..(7): Am6(F)
  misc_feature (9)..(9): Am6(F)
  misc_feature (11)..(12): Am6(F)
  misc_feature (16)..(16): Am6(F)
  misc_feature (31)..(31): Am6(F)
  misc_feature (35)..(35): Am6(F)
gggngnnuncnngcuncuuguucuuuuugcngccnccauggacuacaaggacgacgacgacaagaucaucgacuauaaagacgacgacgauaaagguggcgacuauaaggacgacgacgacaaacaccaccaccaccaccacuga

SEQ ID NO: 63 - RNA, 80 nt, Artificial Sequence
  E21-1
  misc_feature (4)..(4): Am6(F)
  misc_feature (6)..(7): Am6(F)
  misc_feature (9)..(9): Am6(F)
  misc_feature (11)..(12): Am6(F)
  misc_feature (16)..(16): Am6(F)
  misc_feature (31)..(31): Am6(F)
  misc_feature (35)..(35): Am6(F)
gggngnnuncnngcuncuuguucuuuuugcngccnccauggacuacaaggacgacgacgacaagaucaucgacuauaaag

SEQ ID NO: 64 - RNA, 65 nt, Artificial Sequence; identical to SEQ ID NO: 10
  E21-2

SEQ ID NO: 65 - RNA, 145 nt, Artificial Sequence; identical to SEQ ID NO: 62
  E22
  misc_feature (4)..(4): Am6(F)
  misc_feature (6)..(7): Am6(F)
  misc_feature (9)..(9): Am6(F)
  misc_feature (11)..(12): Am6(F)
  misc_feature (16)..(16): Am6(F)
  misc_feature (31)..(31): Am6(F)
  misc_feature (35)..(35): Am6(F)

SEQ ID NO: 66 - RNA, 80 nt, Artificial Sequence; identical to SEQ ID NO: 63
  E22-1
  misc_feature (4)..(4): Am6(F)
  misc_feature (6)..(7): Am6(F)
  misc_feature (9)..(9): Am6(F)
  misc_feature (11)..(12): Am6(F)
  misc_feature (16)..(16): Am6(F)
  misc_feature (31)..(31): Am6(F)
  misc_feature (35)..(35): Am6(F)

SEQ ID NO: 67 - RNA, 65 nt, Artificial Sequence; identical to SEQ ID NO: 10
  E22-2

SEQ ID NO: 68 - RNA, 145 nt, Artificial Sequence; identical to SEQ ID NO: 1
  E23

SEQ ID NO: 69 - RNA, 80 nt, Artificial Sequence; identical to SEQ ID NO: 2
  E23-1

SEQ ID NO: 70 - RNA, 65 nt, Artificial Sequence; identical to SEQ ID NO: 10
  E23-2

SEQ ID NO: 71 - RNA, 145 nt, Artificial Sequence; identical to SEQ ID NO: 62
  E24
  misc_feature (4)..(4): Am6(M)
  misc_feature (6)..(7): Am6(M)
  misc_feature (9)..(9): Am6(M)
  misc_feature (11)..(12): Am6(M)
  misc_feature (16)..(16): Am6(M)
  misc_feature (31)..(31): Am6(M)
  misc_feature (35)..(35): Am6(M)

SEQ ID NO: 72 - RNA, 80 nt, Artificial Sequence; identical to SEQ ID NO: 63
  E24-1
  misc_feature (4)..(4): Am6(M)
  misc_feature (6)..(7): Am6(M)
  misc_feature (9)..(9): Am6(M)
  misc_feature (11)..(12): Am6(M)
  misc_feature (16)..(16): Am6(M)
  misc_feature (31)..(31): Am6(M)
  misc_feature (35)..(35): Am6(M)

SEQ ID NO: 73 - RNA, 65 nt, Artificial Sequence; identical to SEQ ID NO: 10
  E24-2

SEQ ID NO: 74 - RNA, 145 nt, Artificial Sequence; identical to SEQ ID NO: 62
  E25
  misc_feature (4)..(4): Am6(F)
  misc_feature (6)..(7): Am6(F)
  misc_feature (9)..(9): Am6(F)
  misc_feature (11)..(12): Am6(F)
  misc_feature (16)..(16): Am6(F)
  misc_feature (31)..(31): Am6(F)
  misc_feature (35)..(35): Am6(F)

SEQ ID NO: 75 - RNA, 80 nt, Artificial Sequence; identical to SEQ ID NO: 63
  E25-1
  misc_feature (4)..(4): Am6(F)
  misc_feature (6)..(7): Am6(F)
  misc_feature (9)..(9): Am6(F)
  misc_feature (11)..(12): Am6(F)
  misc_feature (16)..(16): Am6(F)
  misc_feature (31)..(31): Am6(F)
  misc_feature (35)..(35): Am6(F)

SEQ ID NO: 76 - RNA, 65 nt, Artificial Sequence; identical to SEQ ID NO: 10
  E25-2

SEQ ID NO: 77 - RNA, 165 nt, Artificial Sequence; identical to SEQ ID NO: 11
  E26

SEQ ID NO: 78 - RNA, 80 nt, Artificial Sequence; identical to SEQ ID NO: 2
  E26-1

SEQ ID NO: 79 - RNA, 85 nt, Artificial Sequence; identical to SEQ ID NO: 13
  E26-2

SEQ ID NO: 80 - RNA, 165 nt, Artificial Sequence; identical to SEQ ID NO: 11
  E27

SEQ ID NO: 81 - RNA, 80 nt, Artificial Sequence; identical to SEQ ID NO: 2
  E27-1

SEQ ID NO: 82 - RNA, 85 nt, Artificial Sequence; identical to SEQ ID NO: 13
  E27-2

SEQ ID NO: 83 - RNA, 165 nt, Artificial Sequence; identical to SEQ ID NO: 11
  E28

SEQ ID NO: 84 - RNA, 80 nt, Artificial Sequence; identical to SEQ ID NO: 2
  E28-1

SEQ ID NO: 85 - RNA, 85 nt, Artificial Sequence; identical to SEQ ID NO: 13
  E28-2

SEQ ID NO: 86 - RNA, 165 nt, Artificial Sequence; identical to SEQ ID NO: 11
  E29

SEQ ID NO: 87 - RNA, 80 nt, Artificial Sequence; identical to SEQ ID NO: 2
  E29-1

SEQ ID NO: 88 - RNA, 85 nt, Artificial Sequence; identical to SEQ ID NO: 13
  E29-2

SEQ ID NO: 89 - RNA, 91 nt, Artificial Sequence
  E30
gggagaauacaagcuacuuguucuuuuugcagccaccauggacuauaaggacgacgacgacaaagguggccaccaccaccaccaccacuga

SEQ ID NO: 90 - RNA, 91 nt, Artificial Sequence; identical to SEQ ID NO: 89
  E31

SEQ ID NO: 91 - RNA, 145 nt, Artificial Sequence; identical to SEQ ID NO: 1
  E32

SEQ ID NO: 92 - RNA, 80 nt, Artificial Sequence; identical to SEQ ID NO: 2
  32-1

SEQ ID NO: 93 - RNA, 65 nt, Artificial Sequence; identical to SEQ ID NO: 10
  E32-2

SEQ ID NO: 94 - RNA, 145 nt, Artificial Sequence; identical to SEQ ID NO: 1
  E33

SEQ ID NO: 95 - RNA, 80 nt, Artificial Sequence; identical to SEQ ID NO: 2
  E33-1

SEQ ID NO: 96 - RNA, 65 nt, Artificial Sequence; identical to SEQ ID NO: 10
  E33-2

SEQ ID NO: 97 - RNA, 145 nt, Artificial Sequence; identical to SEQ ID NO: 1
  E34

SEQ ID NO: 98 - RNA, 65 nt, Artificial Sequence; identical to SEQ ID NO: 10
  E34-1

SEQ ID NO: 99 - RNA, 65 nt, Artificial Sequence; identical to SEQ ID NO: 10
  E34-2

SEQ ID NO: 100 - RNA, 145 nt, Artificial Sequence; identical to SEQ ID NO: 1
  E35

SEQ ID NO: 101 - RNA, 80 nt, Artificial Sequence; identical to SEQ ID NO: 2
  E35-1

SEQ ID NO: 102 - RNA, 65 nt, Artificial Sequence; identical to SEQ ID NO: 10
  E35-2

SEQ ID NO: 103 - RNA, 145 nt, Artificial Sequence; identical to SEQ ID NO: 1
  E36

SEQ ID NO: 104 - RNA, 80 nt, Artificial Sequence; identical to SEQ ID NO: 2
  E36-1

SEQ ID NO: 105 - RNA, 65 nt, Artificial Sequence; identical to SEQ ID NO: 10
  E36-2

SEQ ID NO: 106 - RNA, 145 nt, Artificial Sequence; identical to SEQ ID NO: 1
  E37

SEQ ID NO: 107 - RNA, 80 nt, Artificial Sequence; identical to SEQ ID NO: 2
  E37-1

SEQ ID NO: 108 - RNA, 65 nt, Artificial Sequence; identical to SEQ ID NO: 10
  E37-2

SEQ ID NO: 109 - RNA, 145 nt, Artificial Sequence; identical to SEQ ID NO: 1
  E38

SEQ ID NO: 110 - RNA, 80 nt, Artificial Sequence; identical to SEQ ID NO: 2
  E38-1

SEQ ID NO: 111 - RNA, 65 nt, Artificial Sequence; identical to SEQ ID NO: 10
  E38-2

SEQ ID NO: 112 - RNA, 145 nt, Artificial Sequence; identical to SEQ ID NO: 1
  E39

SEQ ID NO: 113 - RNA, 80 nt, Artificial Sequence; identical to SEQ ID NO: 2
  E39-1

SEQ ID NO: 114 - RNA, 65 nt, Artificial Sequence; identical to SEQ ID NO: 10
  E39-2

SEQ ID NO: 115 - RNA, 145 nt, Artificial Sequence; identical to SEQ ID NO: 1
  E40

SEQ ID NO: 116 - RNA, 80 nt, Artificial Sequence; identical to SEQ ID NO: 2
  E40-1

SEQ ID NO: 117 - RNA, 65 nt, Artificial Sequence; identical to SEQ ID NO: 10
  E40-2

SEQ ID NO: 118 - RNA, 145 nt, Artificial Sequence; identical to SEQ ID NO: 1
  E41

SEQ ID NO: 119 - RNA, 80 nt, Artificial Sequence; identical to SEQ ID NO: 2
  E41-1

SEQ ID NO: 120 - RNA, 65 nt, Artificial Sequence; identical to SEQ ID NO: 10
  E41-2

SEQ ID NO: 121 - RNA, 145 nt, Artificial Sequence; identical to SEQ ID NO: 1
  E42

SEQ ID NO: 122 - RNA, 80 nt, Artificial Sequence; identical to SEQ ID NO: 2
  42-1

SEQ ID NO: 123 - RNA, 65 nt, Artificial Sequence; identical to SEQ ID NO: 10
  42-2

SEQ ID NO: 124 - RNA, 145 nt, Artificial Sequence; identical to SEQ ID NO: 1
  E43

SEQ ID NO: 125 - RNA, 80 nt, Artificial Sequence; identical to SEQ ID NO: 2
  E43-1

SEQ ID NO: 126 - RNA, 65 nt, Artificial Sequence; identical to SEQ ID NO: 10
  E43-2

SEQ ID NO: 127 - RNA, 145 nt, Artificial Sequence; identical to SEQ ID NO: 1
  E44

SEQ ID NO: 128 - RNA, 80 nt, Artificial Sequence; identical to SEQ ID NO: 2
  E44-1

SEQ ID NO: 129 - RNA, 65 nt, Artificial Sequence; identical to SEQ ID NO: 10
  E44-2

SEQ ID NO: 130 - RNA, 165 nt, Artificial Sequence; identical to SEQ ID NO: 11
  E45

SEQ ID NO: 131 - RNA, 80 nt, Artificial Sequence; identical to SEQ ID NO: 2
  E45-1

SEQ ID NO: 132 - RNA, 85 nt, Artificial Sequence; identical to SEQ ID NO: 13
  E45-2

SEQ ID NO: 133 - RNA, 165 nt, Artificial Sequence; identical to SEQ ID NO: 11
  E46

SEQ ID NO: 134 - RNA, 80 nt, Artificial Sequence; identical to SEQ ID NO: 2
  E46-1

SEQ ID NO: 135 - RNA, 85 nt, Artificial Sequence; identical to SEQ ID NO: 13
  E46-2

SEQ ID NO: 136 - DNA, 145 bp, Artificial Sequence
  E47
gggagaauacaagcuacuuguucuuuuugcagccaccauggacuacaaggacgacgacgacaagaucaucgacuauaaagacgacgacgauaaagguggcgacuauaaggacgacgacgacaaacaccaccaccaccaccactga

SEQ ID NO: 137 - DNA, 145 bp, Artificial Sequence; identical to SEQ ID NO: 136
  E38

SEQ ID NO: 138 - DNA, 145 bp, Artificial Sequence; identical to SEQ ID NO: 136
  E49

SEQ ID NO: 139 - DNA, 145 bp, Artificial Sequence; identical to SEQ ID NO: 136
  E50

SEQ ID NO: 140 - DNA, 149 bp, Artificial Sequence
  E51
  misc_feature (20)..(20): rSpacer
  misc_feature (23)..(23): rSpacer
  misc_feature (26)..(26): rSpacer
  misc_feature (29)..(29): rSpacer
gggagaauacaagcuacuungunucnuunuuugcagccaccauggacuacaaggacgacgacgacaagaucaucgacuauaaagacgacgacgauaaagguggcgacuauaaggacgacgacgacaaacaccaccaccaccaccactga

SEQ ID NO: 141 - RNA, 84 nt, Artificial Sequence
  E51-1
  misc_feature (20)..(20): rSpacer
  misc_feature (23)..(23): rSpacer
  misc_feature (26)..(26): rSpacer
  misc_feature (29)..(29): rSpacer
gggagaauacaagcuacuungunucnuunuuugcagccaccauggacuacaaggacgacgacgacaagaucaucgacuauaaag

SEQ ID NO: 142 - DNA, 65 bp, Artificial Sequence
  E51-2
acgacgacgauaaagguggcgacuauaaggacgacgacgacaaacaccaccaccaccaccactga

SEQ ID NO: 143 - DNA, 145 bp, Artificial Sequence; identical to SEQ ID NO: 136
  E52

SEQ ID NO: 144 - RNA, 80 nt, Artificial Sequence; identical to SEQ ID NO: 2
  E52-1

SEQ ID NO: 145 - DNA, 65 bp, Artificial Sequence; identical to SEQ ID NO: 142
  E52-2

SEQ ID NO: 146 - DNA, 165 bp, Artificial Sequence; identical to SEQ ID NO: 5
  E53

SEQ ID NO: 147 - RNA, 80 nt, Artificial Sequence; identical to SEQ ID NO: 2
  E53-1

SEQ ID NO: 148 - DNA, 85 bp, Artificial Sequence; identical to SEQ ID NO: 7
  E53-2

SEQ ID NO: 149 - DNA, 165 bp, Artificial Sequence; identical to SEQ ID NO: 5
  E54

SEQ ID NO: 150 - RNA, 80 nt, Artificial Sequence; identical to SEQ ID NO: 2
  E54-1

SEQ ID NO: 151 - DNA, 85 bp, Artificial Sequence; identical to SEQ ID NO: 7
  E54-2

SEQ ID NO: 152 - DNA, 165 bp, Artificial Sequence; identical to SEQ ID NO: 5
  E55

SEQ ID NO: 153 - RNA, 80 nt, Artificial Sequence; identical to SEQ ID NO: 2
  E55-1

SEQ ID NO: 154 - DNA, 85 bp, Artificial Sequence; identical to SEQ ID NO: 7
  E55-2

SEQ ID NO: 155 - DNA, 165 bp, Artificial Sequence; identical to SEQ ID NO: 5
  E56

SEQ ID NO: 156 - RNA, 80 nt, Artificial Sequence; identical to SEQ ID NO: 2
  E56-1

SEQ ID NO: 157 - DNA, 85 bp, Artificial Sequence; identical to SEQ ID NO: 7
  E56-2

SEQ ID NO: 158 - DNA, 165 bp, Artificial Sequence; identical to SEQ ID NO: 5
  E57

SEQ ID NO: 159 - RNA, 80 nt, Artificial Sequence; identical to SEQ ID NO: 2
  E57-1

SEQ ID NO: 160 - DNA, 85 bp, Artificial Sequence; identical to SEQ ID NO: 7
  E57-2

SEQ ID NO: 161 - DNA, 185 bp, Artificial Sequence
  E58
gggagaauacaagcuacuuguucuuuuugcagccaccauggacuacaaggacgacgacgacaagaucaucgacuauaaagacgacgacgauaaagguggcgacuauaaggacgacgacgacaaacaccaccaccaccaccactgaaaaaaaaaaaaaaaaaaaaaaaaaaaaaaaaaaaaaaaaa

SEQ ID NO: 162 - RNA, 80 nt, Artificial Sequence; identical to SEQ ID NO: 2
  E58-1

SEQ ID NO: 163 - DNA, 105 bp, Artificial Sequence
  E58-2
acgacgacgauaaagguggcgacuauaaggacgacgacgacaaacaccaccaccaccaccactgaaaaaaaaaaaaaaaaaaaaaaaaaaaaaaaaaaaaaaaaa

SEQ ID NO: 164 - DNA, 185 bp, Artificial Sequence; identical to SEQ ID NO: 161
  E59

SEQ ID NO: 165 - RNA, 80 nt, Artificial Sequence; identical to SEQ ID NO: 2
  E59-1

SEQ ID NO: 166 - DNA, 105 bp, Artificial Sequence; identical to SEQ ID NO: 163
  E59-2

SEQ ID NO: 167 - DNA, 165 bp, Artificial Sequence; identical to SEQ ID NO: 5
  E60

SEQ ID NO: 168 - DNA, 80 bp, Artificial Sequence
  E60-1
gggagaauacaagcuacuuguucuuuuugcagccaccauggacuacaaggacgacgacgacaagaucaucgacuauaaag

SEQ ID NO: 169 - DNA, 85 bp, Artificial Sequence; identical to SEQ ID NO: 7
  E60-2

SEQ ID NO: 170 - RNA, 91 nt, Artificial Sequence; identical to SEQ ID NO: 89
  E61

SEQ ID NO: 171 - DNA, 165 bp, Artificial Sequence; identical to SEQ ID NO: 5
  E62

SEQ ID NO: 172 - RNA, 80 nt, Artificial Sequence; identical to SEQ ID NO: 2
  E62-1

SEQ ID NO: 173 - DNA, 85 bp, Artificial Sequence; identical to SEQ ID NO: 7
  E62-2

SEQ ID NO: 174 - DNA, 165 bp, Artificial Sequence; identical to SEQ ID NO: 5
  E63-1

SEQ ID NO: 175 - RNA, 80 nt, Artificial Sequence; identical to SEQ ID NO: 2
  E63-1

SEQ ID NO: 176 - DNA, 85 bp, Artificial Sequence; identical to SEQ ID NO: 7
  E63-2

SEQ ID NO: 177 - DNA, 165 bp, Artificial Sequence; identical to SEQ ID NO: 5
  E64

SEQ ID NO: 178 - RNA, 80 nt, Artificial Sequence; identical to SEQ ID NO: 2
  E64-1

SEQ ID NO: 179 - DNA, 85 bp, Artificial Sequence; identical to SEQ ID NO: 7
  E64-2

SEQ ID NO: 180 - DNA, 165 bp, Artificial Sequence; identical to SEQ ID NO: 5
  E65

SEQ ID NO: 181 - RNA, 80 nt, Artificial Sequence; identical to SEQ ID NO: 2
  E65-1

SEQ ID NO: 182 - DNA, 85 bp, Artificial Sequence; identical to SEQ ID NO: 7
  E65-2

SEQ ID NO: 183 - DNA, 165 bp, Artificial Sequence; identical to SEQ ID NO: 5
  E66

SEQ ID NO: 184 - RNA, 80 nt, Artificial Sequence; identical to SEQ ID NO: 2
  E66-1

SEQ ID NO: 185 - DNA, 85 bp, Artificial Sequence; identical to SEQ ID NO: 7
  E66-2

SEQ ID NO: 186 - DNA, 165 bp, Artificial Sequence; identical to SEQ ID NO: 5
  E67

SEQ ID NO: 187 - RNA, 80 nt, Artificial Sequence; identical to SEQ ID NO: 2
  E67-1

SEQ ID NO: 188 - DNA, 85 bp, Artificial Sequence; identical to SEQ ID NO: 7
  E67-2

SEQ ID NO: 189 - DNA, 165 bp, Artificial Sequence; identical to SEQ ID NO: 5
  E68

SEQ ID NO: 190 - RNA, 80 nt, Artificial Sequence; identical to SEQ ID NO: 2
  E68-1

SEQ ID NO: 191 - DNA, 85 bp, Artificial Sequence; identical to SEQ ID NO: 7
  E68-2

SEQ ID NO: 192 - RNA, 165 nt, Artificial Sequence; identical to SEQ ID NO: 11
  E69

SEQ ID NO: 193 - RNA, 80 nt, Artificial Sequence; identical to SEQ ID NO: 2
  E69-1

SEQ ID NO: 194 - RNA, 85 nt, Artificial Sequence; identical to SEQ ID NO: 13
  E69-2

SEQ ID NO: 195 - RNA, 165 nt, Artificial Sequence; identical to SEQ ID NO: 11
  E70

SEQ ID NO: 196 - RNA, 80 nt, Artificial Sequence; identical to SEQ ID NO: 2
  E70-1

SEQ ID NO: 197 - RNA, 85 nt, Artificial Sequence; identical to SEQ ID NO: 13
  E70-2

SEQ ID NO: 198 - DNA, 91 bp, Artificial Sequence
  E71
gggagaauacaagcuacuuguucuuuuugcagccaccauggacuauaaggacgacgacgacaaagguggccaccaccaccaccaccactga

SEQ ID NO: 199 - DNA, 91 bp, Artificial Sequence
  E72
  misc_feature (19)..(19): rSpacer
  misc_feature (21)..(21): rSpacer
  misc_feature (23)..(23): rSpacer
  misc_feature (25)..(25): rSpacer
gggagaauacaagcuacungnununuuugcagccaccauggacuauaaggacgacgacgacaaagguggccaccaccaccaccaccactga

SEQ ID NO: 200 - DNA, 91 bp, Artificial Sequence; identical to SEQ ID NO: 199
  E73
  misc_feature (19)..(19): dSpacer
  misc_feature (21)..(21): dSpacer
  misc_feature (23)..(23): dSpacer
  misc_feature (25)..(25): dSpacer

SEQ ID NO: 201 - DNA, 91 bp, Artificial Sequence; identical to SEQ ID NO: 199
  E74
  misc_feature (19)..(19): C3
  misc_feature (21)..(21): C3
  misc_feature (23)..(23): C3
  misc_feature (25)..(25): C3

SEQ ID NO: 202 - DNA, 91 bp, Artificial Sequence; identical to SEQ ID NO: 199
  E75
  misc_feature (19)..(19): Pyrrolidine
  misc_feature (21)..(21): Pyrrolidine
  misc_feature (23)..(23): Pyrrolidine
  misc_feature (25)..(25): Pyrrolidine

SEQ ID NO: 203 - DNA, 91 bp, Artificial Sequence; identical to SEQ ID NO: 199
  E76
  misc_feature (19)..(19): Ethynyl-dSpacer
  misc_feature (21)..(21): Ethynyl-dSpacer
  misc_feature (23)..(23): Ethynyl-dSpacer
  misc_feature (25)..(25): Ethynyl-dSpacer

SEQ ID NO: 204 - DNA, 91 bp, Artificial Sequence
  E77
  misc_feature (9)..(9): rSpacer
  misc_feature (11)..(11): rSpacer
  misc_feature (13)..(13): rSpacer
  misc_feature (15)..(15): rSpacer
gggagaauncnancnacuuguucuuuuugcagccaccauggacuauaaggacgacgacgacaaagguggccaccaccaccaccaccactga

SEQ ID NO: 205 - DNA, 91 bp, Artificial Sequence
  E78
  misc_feature (28)..(28): rSpacer
  misc_feature (30)..(30): rSpacer
  misc_feature (32)..(32): rSpacer
  misc_feature (34)..(34): rSpacer
gggagaauacaagcuacuuguucuuuungnancnaccauggacuauaaggacgacgacgacaaagguggccaccaccaccaccaccactga

SEQ ID NO: 206 - DNA, 165 bp, Artificial Sequence; identical to SEQ ID NO: 5
  E79

SEQ ID NO: 207 - RNA, 80 nt, Artificial Sequence; identical to SEQ ID NO: 2
  E79-1

SEQ ID NO: 208 - DNA, 85 bp, Artificial Sequence; identical to SEQ ID NO: 7
  E79-2

SEQ ID NO: 209 - DNA, 165 bp, Artificial Sequence; identical to SEQ ID NO: 5
  E80

SEQ ID NO: 210 - RNA, 80 nt, Artificial Sequence; identical to SEQ ID NO: 2
  E80-1

SEQ ID NO: 211 - DNA, 85 bp, Artificial Sequence; identical to SEQ ID NO: 7
  E80-2

SEQ ID NO: 212 - DNA, 165 bp, Artificial Sequence; identical to SEQ ID NO: 5
  E81

SEQ ID NO: 213 - RNA, 80 nt, Artificial Sequence; identical to SEQ ID NO: 2
  E81-1

SEQ ID NO: 214 - DNA, 85 bp, Artificial Sequence; identical to SEQ ID NO: 7
  E81-4

SEQ ID NO: 215 - DNA, 165 bp, Artificial Sequence; identical to SEQ ID NO: 5
  E82

SEQ ID NO: 216 - RNA, 80 nt, Artificial Sequence; identical to SEQ ID NO: 2
  E82-1

SEQ ID NO: 217 - DNA, 85 bp, Artificial Sequence; identical to SEQ ID NO: 7
  E82-2

SEQ ID NO: 218 - DNA, 165 bp, Artificial Sequence; identical to SEQ ID NO: 5
  E83

SEQ ID NO: 219 - RNA, 80 nt, Artificial Sequence; identical to SEQ ID NO: 2
  E83-1

SEQ ID NO: 220 - DNA, 85 bp, Artificial Sequence; identical to SEQ ID NO: 7
  E83-2

SEQ ID NO: 221 - DNA, 165 bp, Artificial Sequence; identical to SEQ ID NO: 5
  E84

SEQ ID NO: 222 - DNA, 80 bp, Artificial Sequence; identical to SEQ ID NO: 168
  E84-1

SEQ ID NO: 223 - DNA, 85 bp, Artificial Sequence; identical to SEQ ID NO: 7
  E84-2

SEQ ID NO: 224 - DNA, 91 bp, Artificial Sequence; identical to SEQ ID NO: 198
  E85

SEQ ID NO: 225 - DNA, 91 bp, Artificial Sequence; identical to SEQ ID NO: 199
  E86
  misc_feature (19)..(19): rSpacer
  misc_feature (21)..(21): rSpacer
  misc_feature (23)..(23): rSpacer
  misc_feature (25)..(25): rSpacer

SEQ ID NO: 226 - DNA, 91 bp, Artificial Sequence; identical to SEQ ID NO: 198
  E87

SEQ ID NO: 227 - DNA, 91 bp, Artificial Sequence
  E88
  misc_feature (18)..(18): rSpacer
  misc_feature (20)..(20): rSpacer
  misc_feature (22)..(22): rSpacer
  misc_feature (24)..(24): rSpacer
gggagaauacaagcuacnununcnuuuugcagccaccauggacuauaaggacgacgacgacaaagguggccaccaccaccaccaccactga

SEQ ID NO: 228 - DNA, 91 bp, Artificial Sequence
  E89
  misc_feature (9)..(9): rSpacer
  misc_feature (11)..(11): rSpacer
  misc_feature (13)..(13): rSpacer
  misc_feature (15)..(15): rSpacer
  misc_feature (19)..(19): rSpacer
  misc_feature (21)..(21): rSpacer
  misc_feature (23)..(23): rSpacer
  misc_feature (25)..(25): rSpacer
gggagaauncnancnacungnununuuugcagccaccauggacuauaaggacgacgacgacaaagguggccaccaccaccaccaccactga

SEQ ID NO: 229 - DNA, 91 bp, Artificial Sequence
  E90
  misc_feature (18)..(25): rSpacer
gggagaauacaagcuacnnnnnnnnuuugcagccaccauggacuauaaggacgacgacgacaaagguggccaccaccaccaccaccactga

SEQ ID NO: 230 - DNA, 91 bp, Artificial Sequence
  E91
  misc_feature (7)..(7): rSpacer
  misc_feature (9)..(9): rSpacer
  misc_feature (11)..(11): rSpacer
  misc_feature (13)..(13): rSpacer
  misc_feature (15)..(15): rSpacer
  misc_feature (17)..(17): rSpacer
  misc_feature (19)..(19): rSpacer
  misc_feature (21)..(21): rSpacer
  misc_feature (23)..(23): rSpacer
  misc_feature (25)..(25): n is a, c, g, t or u
  misc_feature (27)..(27): rSpacer
  misc_feature (29)..(29): rSpacer
gggaganuncnancnanungnununununcagccaccauggacuauaaggacgacgacgacaaagguggccaccaccaccaccaccactga

SEQ ID NO: 231 - DNA, 91 bp, Artificial Sequence
  E92
  misc_feature (8)..(8): rSpacer
  misc_feature (10)..(10): rSpacer
  misc_feature (12)..(12): rSpacer
  misc_feature (14)..(14): rSpacer
  misc_feature (16)..(16): rSpacer
  misc_feature (18)..(18): rSpacer
  misc_feature (20)..(20): rSpacer
  misc_feature (22)..(22): rSpacer
  misc_feature (24)..(24): rSpacer
  misc_feature (26)..(26): rSpacer
  misc_feature (28)..(28): rSpacer
  misc_feature (30)..(30): rSpacer
gggagaananangnuncnununcnunungnagccaccauggacuauaaggacgacgacgacaaagguggccaccaccaccaccaccactga

SEQ ID NO: 232 - DNA, 91 bp, Artificial Sequence; identical to SEQ ID NO: 198
  E93

SEQ ID NO: 233 - DNA, 91 bp, Artificial Sequence; identical to SEQ ID NO: 198
  E94

SEQ ID NO: 234 - DNA, 165 bp, Artificial Sequence; identical to SEQ ID NO: 5
  E95

SEQ ID NO: 235 - RNA, 80 nt, Artificial Sequence; identical to SEQ ID NO: 2
  E95-1

SEQ ID NO: 236 - DNA, 85 bp, Artificial Sequence; identical to SEQ ID NO: 7
  E95-2

SEQ ID NO: 237 - RNA, 91 nt, Artificial Sequence; identical to SEQ ID NO: 89
  E96

SEQ ID NO: 238 - RNA, 91 nt, Artificial Sequence; identical to SEQ ID NO: 89
  E97

SEQ ID NO: 239 - DNA, 91 bp, Artificial Sequence; identical to SEQ ID NO: 198
  E98

SEQ ID NO: 240 - DNA, 91 bp, Artificial Sequence; identical to SEQ ID NO: 198
  E99

SEQ ID NO: 241 - DNA, 91 bp, Artificial Sequence; identical to SEQ ID NO: 198
  E100

SEQ ID NO: 242 - DNA, 91 bp, Artificial Sequence; identical to SEQ ID NO: 198
  E101

SEQ ID NO: 243 - DNA, 91 bp, Artificial Sequence; identical to SEQ ID NO: 198
  E102

SEQ ID NO: 244 - DNA, 91 bp, Artificial Sequence; identical to SEQ ID NO: 198
  E103

SEQ ID NO: 245 - DNA, 91 bp, Artificial Sequence
  E104
  misc_feature (8)..(8): rSpacer
  misc_feature (11)..(11): rSpacer
  misc_feature (14)..(14): rSpacer
  misc_feature (17)..(17): rSpacer
  misc_feature (20)..(20): rSpacer
  misc_feature (23)..(23): rSpacer
  misc_feature (26)..(26): rSpacer
gggagaanacnagnuanuunuunuunuugcagccaccauggacuauaaggacgacgacgacaaagguggccaccaccaccaccaccactga

SEQ ID NO: 246 - DNA, 91 bp, Artificial Sequence
  E105
  misc_feature (32)..(32): rSpacer
  misc_feature (35)..(35): rSpacer
gggagaauacaagcuacuuguucuuuuugcanccnccauggacuauaaggacgacgacgacaaagguggccaccaccaccaccaccactga

SEQ ID NO: 247 - DNA, 91 bp, Artificial Sequence; identical to SEQ ID NO: 245
  E106
  misc_feature (8)..(8): dSpacer
  misc_feature (11)..(11): dSpacer
  misc_feature (14)..(14): dSpacer
  misc_feature (17)..(17): dSpacer
  misc_feature (20)..(20): dSpacer
  misc_feature (23)..(23): dSpacer
  misc_feature (26)..(26): dSpacer

SEQ ID NO: 248 - DNA, 91 bp, Artificial Sequence; identical to SEQ ID NO: 246
  E107
  misc_feature (32)..(32): dSpacer
  misc_feature (35)..(35): dSpacer

SEQ ID NO: 249 - DNA, 91 bp, Artificial Sequence; identical to SEQ ID NO: 245
  E108
  misc_feature (8)..(8): C3
  misc_feature (11)..(11): C3
  misc_feature (14)..(14): C3
  misc_feature (17)..(17): C3
  misc_feature (20)..(20): C3
  misc_feature (23)..(23): C3
  misc_feature (26)..(26): C3

SEQ ID NO: 250 - DNA, 91 bp, Artificial Sequence; identical to SEQ ID NO: 246
  E109
  misc_feature (32)..(32): C2
  misc_feature (35)..(35): C2

SEQ ID NO: 251 - DNA, 91 bp, Artificial Sequence; identical to SEQ ID NO: 198
  E110

SEQ ID NO: 252 - DNA, 91 bp, Artificial Sequence; identical to SEQ ID NO: 198
  E111

SEQ ID NO: 253 - DNA, 91 bp, Artificial Sequence; identical to SEQ ID NO: 198
  E112

SEQ ID NO: 254 - DNA, 91 bp, Artificial Sequence; identical to SEQ ID NO: 198
  E113

SEQ ID NO: 255 - DNA, 91 bp, Artificial Sequence; identical to SEQ ID NO: 198
  E114

SEQ ID NO: 256 - DNA, 91 bp, Artificial Sequence; identical to SEQ ID NO: 198
  E115

SEQ ID NO: 257 - DNA, 91 bp, Artificial Sequence
  E116
gggagaatacaagcuacuuguucuutuugcagccaccauggacuauaaggacgacgacgacaaagguggccaccaccaccaccaccactga

SEQ ID NO: 258 - DNA, 91 bp, Artificial Sequence
  E117
gggagaauacaagctactugtuctuutugcagccaccauggacuauaaggacgacgacgacaaagguggccaccaccaccaccaccactga

SEQ ID NO: 259 - DNA, 91 bp, Artificial Sequence
  E118
gggagaauacaagcuacutgutcutuutgcagccaccauggacuauaaggacgacgacgacaaagguggccaccaccaccaccaccactga

SEQ ID NO: 260 - DNA, 91 bp, Artificial Sequence; identical to SEQ ID NO: 257
  E119

SEQ ID NO: 261 - DNA, 91 bp, Artificial Sequence; identical to SEQ ID NO: 257
  E120

SEQ ID NO: 262 - DNA, 91 bp, Artificial Sequence; identical to SEQ ID NO: 245
  E121
  misc_feature (8)..(8): rSpacer
  misc_feature (11)..(11): rSpacer
  misc_feature (14)..(14): rSpacer
  misc_feature (17)..(17): rSpacer
  misc_feature (20)..(20): rSpacer
  misc_feature (23)..(23): rSpacer
  misc_feature (26)..(26): rSpacer

SEQ ID NO: 263 - DNA, 91 bp, Artificial Sequence; identical to SEQ ID NO: 246
  E122
  misc_feature (32)..(32): rSpacer
  misc_feature (35)..(35): rSpacer

SEQ ID NO: 264 - DNA, 91 bp, Artificial Sequence; identical to SEQ ID NO: 245
  E123
  misc_feature (8)..(8): dSpacer
  misc_feature (11)..(11): dSpacer
  misc_feature (14)..(14): dSpacer
  misc_feature (17)..(17): dSpacer
  misc_feature (20)..(20): dSpacer
  misc_feature (23)..(23): dSpacer
  misc_feature (26)..(26): dSpacer

SEQ ID NO: 265 - DNA, 91 bp, Artificial Sequence; identical to SEQ ID NO: 245
  E124
  misc_feature (8)..(8): C2
  misc_feature (11)..(11): C2
  misc_feature (14)..(14): C2
  misc_feature (17)..(17): C2
  misc_feature (20)..(20): C2
  misc_feature (23)..(23): C2
  misc_feature (26)..(26): C2

SEQ ID NO: 266 - DNA, 91 bp, Artificial Sequence; identical to SEQ ID NO: 198
  E125

SEQ ID NO: 267 - DNA, 91 bp, Artificial Sequence; identical to SEQ ID NO: 198
  E126

SEQ ID NO: 268 - DNA, 91 bp, Artificial Sequence; identical to SEQ ID NO: 198
  E127

SEQ ID NO: 269 - DNA, 91 bp, Artificial Sequence; identical to SEQ ID NO: 198
  E128

SEQ ID NO: 270 - DNA, 91 bp, Artificial Sequence; identical to SEQ ID NO: 198
  E129

SEQ ID NO: 271 - DNA, 91 bp, Artificial Sequence; identical to SEQ ID NO: 198
  E130

SEQ ID NO: 272 - DNA, 91 bp, Artificial Sequence; identical to SEQ ID NO: 198
  E131

SEQ ID NO: 273 - DNA, 91 bp, Artificial Sequence; identical to SEQ ID NO: 198
  E132

SEQ ID NO: 274 - DNA, 91 bp, Artificial Sequence; identical to SEQ ID NO: 198
  E133

SEQ ID NO: 275 - DNA, 91 bp, Artificial Sequence; identical to SEQ ID NO: 198
  E134

SEQ ID NO: 276 - DNA, 91 bp, Artificial Sequence; identical to SEQ ID NO: 198
  E135

SEQ ID NO: 277 - DNA, 91 bp, Artificial Sequence; identical to SEQ ID NO: 198
  E136

SEQ ID NO: 278 - DNA, 91 bp, Artificial Sequence; identical to SEQ ID NO: 198
  E137

SEQ ID NO: 279 - DNA, 91 bp, Artificial Sequence; identical to SEQ ID NO: 198
  E138

SEQ ID NO: 280 - DNA, 91 bp, Artificial Sequence; identical to SEQ ID NO: 198
  E139

SEQ ID NO: 281 - DNA, 91 bp, Artificial Sequence; identical to SEQ ID NO: 198
  E140

SEQ ID NO: 282 - DNA, 91 bp, Artificial Sequence; identical to SEQ ID NO: 245
  E141
  misc_feature (8)..(8): rSpacer
  misc_feature (11)..(11): rSpacer
  misc_feature (14)..(14): rSpacer
  misc_feature (17)..(17): rSpacer
  misc_feature (20)..(20): rSpacer
  misc_feature (23)..(23): rSpacer
  misc_feature (26)..(26): rSpacer

SEQ ID NO: 283 - DNA, 91 bp, Artificial Sequence; identical to SEQ ID NO: 245
  E142
  misc_feature (8)..(8): rSpacer
  misc_feature (11)..(11): rSpacer
  misc_feature (14)..(14): rSpacer
  misc_feature (17)..(17): rSpacer
  misc_feature (20)..(20): rSpacer
  misc_feature (23)..(23): rSpacer
  misc_feature (26)..(26): rSpacer

SEQ ID NO: 284 - DNA, 91 bp, Artificial Sequence; identical to SEQ ID NO: 245
  E183
  misc_feature (8)..(8): dSpacer
  misc_feature (11)..(11): dSpacer
  misc_feature (14)..(14): dSpacer
  misc_feature (17)..(17): dSpacer
  misc_feature (20)..(20): dSpacer
  misc_feature (23)..(23): dSpacer
  misc_feature (26)..(26): dSpacer

SEQ ID NO: 285 - DNA, 91 bp, Artificial Sequence; identical to SEQ ID NO: 245
  E144
  misc_feature (8)..(8): C2
  misc_feature (11)..(11): C2
  misc_feature (14)..(14): C2
  misc_feature (17)..(17): C2
  misc_feature (20)..(20): C2
  misc_feature (23)..(23): C2
  misc_feature (26)..(26): C2

SEQ ID NO: 286 - DNA, 91 bp, Artificial Sequence; identical to SEQ ID NO: 198
  E145

SEQ ID NO: 287 - DNA, 91 bp, Artificial Sequence; identical to SEQ ID NO: 198
  E146

SEQ ID NO: 288 - DNA, 91 bp, Artificial Sequence; identical to SEQ ID NO: 198
  E147

SEQ ID NO: 289 - DNA, 91 bp, Artificial Sequence; identical to SEQ ID NO: 198
  E148

SEQ ID NO: 290 - DNA, 91 bp, Artificial Sequence; identical to SEQ ID NO: 198
  E149

SEQ ID NO: 291 - DNA, 91 bp, Artificial Sequence; identical to SEQ ID NO: 198
  E150

SEQ ID NO: 292 - DNA, 91 bp, Artificial Sequence; identical to SEQ ID NO: 198
  E151

SEQ ID NO: 293 - DNA, 91 bp, Artificial Sequence; identical to SEQ ID NO: 198
  E152

SEQ ID NO: 294 - DNA, 91 bp, Artificial Sequence
  153
gggagaatacaagcuacutgutcuttutgcagccaccauggacuauaaggacgacgacgacaaagguggccaccaccaccaccaccactga

SEQ ID NO: 295 - DNA, 91 bp, Artificial Sequence; identical to SEQ ID NO: 257
  154

SEQ ID NO: 296 - DNA, 91 bp, Artificial Sequence
  E155
gggagaatacaagctactugtuctuttugcagccaccauggacuauaaggacgacgacgacaaagguggccaccaccaccaccaccactga

SEQ ID NO: 297 - DNA, 91 bp, Artificial Sequence
  E156
gggagaatacaagctacttgttctttttgcagccaccauggacuauaaggacgacgacgacaaagguggccaccaccaccaccaccactga

SEQ ID NO: 298 - DNA, 91 bp, Artificial Sequence; identical to SEQ ID NO: 259
  E157

SEQ ID NO: 299 - DNA, 91 bp, Artificial Sequence; identical to SEQ ID NO: 258
  E158

SEQ ID NO: 300 - DNA, 91 bp, Artificial Sequence
  E159
gggagaauacaagctacttgttcttuttgcagccaccauggacuauaaggacgacgacgacaaagguggccaccaccaccaccaccactga

SEQ ID NO: 301 - DNA, 91 bp, Artificial Sequence; identical to SEQ ID NO: 257
  E160

SEQ ID NO: 302 - DNA, 91 bp, Artificial Sequence; identical to SEQ ID NO: 296
  E161

SEQ ID NO: 303 - DNA, 91 bp, Artificial Sequence
  E162
gggagaatacaagcuacuuguucuuguugcagccaccauggacuauaaggacgacgacgacaaagguggccaccaccaccaccaccactga

SEQ ID NO: 304 - DNA, 91 bp, Artificial Sequence; identical to SEQ ID NO: 296
  E163

SEQ ID NO: 305 - DNA, 189 bp, Artificial Sequence
  E164
  misc_feature (20)..(20): rSpacer
  misc_feature (23)..(23): rSpacer
  misc_feature (26)..(26): rSpacer
  misc_feature (29)..(29): rSpacer
gggagaauacaagcuacuungunucnuunuuugcagccaccauggacuacaaggacgacgacgacaagaucaucgacuauaaagacgacgacgauaaagguggcgacuauaaggacgacgacgacaaacaccaccaccaccaccactgaaaaaaaaaaaaaaaaaaaaaaaaaaaaaaaaaaaaaaaaa

SEQ ID NO: 306 - RNA, 84 nt, Artificial Sequence; identical to SEQ ID NO: 141
  E164-1
  misc_feature (20)..(20): rSpacer
  misc_feature (23)..(23): rSpacer
  misc_feature (26)..(26): rSpacer
  misc_feature (29)..(29): rSpacer

SEQ ID NO: 307 - DNA, 105 bp, Artificial Sequence; identical to SEQ ID NO: 163
  E164-2

SEQ ID NO: 308 - DNA, 165 bp, Artificial Sequence; identical to SEQ ID NO: 5
  E165

SEQ ID NO: 309 - RNA, 80 nt, Artificial Sequence; identical to SEQ ID NO: 2
  E165-1

SEQ ID NO: 310 - DNA, 85 bp, Artificial Sequence; identical to SEQ ID NO: 7
  E165-2

SEQ ID NO: 311 - DNA, 165 bp, Artificial Sequence; identical to SEQ ID NO: 5
  E166

SEQ ID NO: 312 - RNA, 80 nt, Artificial Sequence; identical to SEQ ID NO: 2
  E166-1

SEQ ID NO: 313 - DNA, 85 bp, Artificial Sequence; identical to SEQ ID NO: 7
  E166--2

SEQ ID NO: 314 - DNA, 165 bp, Artificial Sequence; identical to SEQ ID NO: 5
  E167

SEQ ID NO: 315 - RNA, 80 nt, Artificial Sequence; identical to SEQ ID NO: 2
  E167-1

SEQ ID NO: 316 - DNA, 85 bp, Artificial Sequence; identical to SEQ ID NO: 7
  E167-2

SEQ ID NO: 317 - DNA, 165 bp, Artificial Sequence; identical to SEQ ID NO: 5
  E168

SEQ ID NO: 318 - RNA, 80 nt, Artificial Sequence; identical to SEQ ID NO: 2
  E168-1

SEQ ID NO: 319 - DNA, 85 bp, Artificial Sequence; identical to SEQ ID NO: 7
  E168-2

SEQ ID NO: 320 - DNA, 165 bp, Artificial Sequence
  E169
  misc_feature (19)..(19): rSpacer
  misc_feature (21)..(21): rSpacer
  misc_feature (23)..(23): rSpacer
  misc_feature (25)..(25): rSpacer
gggagaauacaagcuacungnununuuugcagccaccauggacuacaaggacgacgacgacaagaucaucgacuauaaagacgacgacgauaaagguggcgacuauaaggacgacgacgacaaacaccaccaccaccaccactgaaaaaaaaaaaaaaaaaaaaa

SEQ ID NO: 321 - RNA, 80 nt, Artificial Sequence
  E169-1
  misc_feature (19)..(19): rSpacer
  misc_feature (21)..(21): rSpacer
  misc_feature (23)..(23): rSpacer
  misc_feature (25)..(25): rSpacer
gggagaauacaagcuacungnununuuugcagccaccauggacuacaaggacgacgacgacaagaucaucgacuauaaag

SEQ ID NO: 322 - DNA, 85 bp, Artificial Sequence; identical to SEQ ID NO: 7
  E169-2

SEQ ID NO: 323 - DNA, 165 bp, Artificial Sequence; identical to SEQ ID NO: 320
  E170
  misc_feature (19)..(19): rSpacer
  misc_feature (21)..(21): rSpacer
  misc_feature (23)..(23): rSpacer
  misc_feature (25)..(25): rSpacer

SEQ ID NO: 324 - RNA, 80 nt, Artificial Sequence; identical to SEQ ID NO: 321
  E170-1
  misc_feature (19)..(19): rSpacer
  misc_feature (21)..(21): rSpacer
  misc_feature (23)..(23): rSpacer
  misc_feature (25)..(25): rSpacer

SEQ ID NO: 325 - DNA, 85 bp, Artificial Sequence; identical to SEQ ID NO: 7
  E170-2

SEQ ID NO: 326 - DNA, 165 bp, Artificial Sequence; identical to SEQ ID NO: 5
  E171

SEQ ID NO: 327 - RNA, 80 nt, Artificial Sequence; identical to SEQ ID NO: 2
  E171-1

SEQ ID NO: 328 - DNA, 85 bp, Artificial Sequence; identical to SEQ ID NO: 7
  E171-2

SEQ ID NO: 329 - DNA, 165 bp, Artificial Sequence; identical to SEQ ID NO: 5
  E172

SEQ ID NO: 330 - RNA, 80 nt, Artificial Sequence; identical to SEQ ID NO: 2
  E172-1

SEQ ID NO: 331 - DNA, 85 bp, Artificial Sequence; identical to SEQ ID NO: 7
  E172-2

SEQ ID NO: 332 - DNA, 165 bp, Artificial Sequence; identical to SEQ ID NO: 5
  E173

SEQ ID NO: 333 - RNA, 80 nt, Artificial Sequence; identical to SEQ ID NO: 2
  E173-1

SEQ ID NO: 334 - DNA, 85 bp, Artificial Sequence; identical to SEQ ID NO: 7
  E173-2

SEQ ID NO: 335 - DNA, 165 bp, Artificial Sequence; identical to SEQ ID NO: 320
  E174
  misc_feature (19)..(19): rSpacer
  misc_feature (21)..(21): rSpacer
  misc_feature (23)..(23): rSpacer
  misc_feature (25)..(25): rSpacer

SEQ ID NO: 336 - RNA, 80 nt, Artificial Sequence; identical to SEQ ID NO: 321
  E174-1
  misc_feature (19)..(19): rSpacer
  misc_feature (21)..(21): rSpacer
  misc_feature (23)..(23): rSpacer
  misc_feature (25)..(25): rSpacer

SEQ ID NO: 337 - DNA, 85 bp, Artificial Sequence; identical to SEQ ID NO: 7
  E174-2

SEQ ID NO: 338 - RNA, 165 nt, Artificial Sequence; identical to SEQ ID NO: 11
  E175

SEQ ID NO: 339 - RNA, 165 nt, Artificial Sequence; identical to SEQ ID NO: 11
  E176

SEQ ID NO: 340 - RNA, 165 nt, Artificial Sequence; identical to SEQ ID NO: 11
  E177

SEQ ID NO: 341 - RNA, 165 nt, Artificial Sequence; identical to SEQ ID NO: 11
  E178

SEQ ID NO: 342 - RNA, 165 nt, Artificial Sequence; identical to SEQ ID NO: 11
  E179

SEQ ID NO: 343 - DNA, 165 bp, Artificial Sequence; identical to SEQ ID NO: 5
  E180

SEQ ID NO: 344 - RNA, 80 nt, Artificial Sequence; identical to SEQ ID NO: 2
  E180-1

SEQ ID NO: 345 - DNA, 85 bp, Artificial Sequence; identical to SEQ ID NO: 7
  E180-2

SEQ ID NO: 346 - DNA, 165 bp, Artificial Sequence; identical to SEQ ID NO: 5
  E181

SEQ ID NO: 347 - RNA, 80 nt, Artificial Sequence; identical to SEQ ID NO: 2
  E181-1

SEQ ID NO: 348 - DNA, 85 bp, Artificial Sequence; identical to SEQ ID NO: 7
  E181-2

SEQ ID NO: 349 - RNA, 175 nt, Artificial Sequence
  E182
gggaaauaagagagaaaagaagaguaagaagaaauauaagagccaccauggacuacaaggacgacgacgacaagaucaucgacuauaaagacgacgacgauaaagguggcgacuauaaggacgacgacgacaaacaccaccaccaccaccacugaaaaaaaaaaaaaaaaaaaaa

SEQ ID NO: 350 - DNA, 175 bp, Artificial Sequence
  E183
gggaaauaagagagaaaagaagaguaagaagaaauauaagagccaccauggacuacaaggacgacgacgacaagaucaucgacuauaaagacgacgacgauaaagguggcgacuauaaggacgacgacgacaaacaccaccaccaccaccactgaaaaaaaaaaaaaaaaaaaaa

SEQ ID NO: 351 - RNA, 90 nt, Artificial Sequence
  E183-1
gggaaauaagagagaaaagaagaguaagaagaaauauaagagccaccauggacuacaaggacgacgacgacaagaucaucgacuauaaag

SEQ ID NO: 352 - DNA, 85 bp, Artificial Sequence; identical to SEQ ID NO: 7
  E183-2

SEQ ID NO: 353 - DNA, 175 bp, Artificial Sequence; identical to SEQ ID NO: 350
  E184

SEQ ID NO: 354 - RNA, 90 nt, Artificial Sequence; identical to SEQ ID NO: 351
  E184-1

SEQ ID NO: 355 - DNA, 85 bp, Artificial Sequence; identical to SEQ ID NO: 7
  E184-2

SEQ ID NO: 356 - DNA, 175 bp, Artificial Sequence; identical to SEQ ID NO: 350
  E185

SEQ ID NO: 357 - RNA, 90 nt, Artificial Sequence; identical to SEQ ID NO: 351
  E185-1

SEQ ID NO: 358 - DNA, 85 bp, Artificial Sequence; identical to SEQ ID NO: 7
  E185-2

SEQ ID NO: 359 - RNA, 178 nt, Artificial Sequence
  E186
gggagaccucuucugguccccacagacucagagagaacccaccggccaccauggacuacaaggacgacgacgacaagaucaucgacuauaaagacgacgacgauaaagguggcgacuauaaggacgacgacgacaaacaccaccaccaccaccacugaaaaaaaaaaaaaaaaaaaaa

SEQ ID NO: 360 - DNA, 178 bp, Artificial Sequence
  E187
gggagaccucuucugguccccacagacucagagagaacccaccggccaccauggacuacaaggacgacgacgacaagaucaucgacuauaaagacgacgacgauaaagguggcgacuauaaggacgacgacgacaaacaccaccaccaccaccactgaaaaaaaaaaaaaaaaaaaaa

SEQ ID NO: 361 - RNA, 93 nt, Artificial Sequence
  E187-1
gggagaccucuucugguccccacagacucagagagaacccaccggccaccauggacuacaaggacgacgacgacaagaucaucgacuauaaag

SEQ ID NO: 362 - DNA, 85 bp, Artificial Sequence; identical to SEQ ID NO: 7
  E187-2

SEQ ID NO: 363 - DNA, 178 bp, Artificial Sequence; identical to SEQ ID NO: 360
  E188

SEQ ID NO: 364 - RNA, 93 nt, Artificial Sequence; identical to SEQ ID NO: 361
  E188-1

SEQ ID NO: 365 - DNA, 85 bp, Artificial Sequence; identical to SEQ ID NO: 7
  E188-2

SEQ ID NO: 366 - RNA, 138 nt, Artificial Sequence
  E189
gggagccaccauggacuacaaggacgacgacgacaagaucaucgacuauaaagacgacgacgauaaagguggcgacuauaaggacgacgacgacaaacaccaccaccaccaccacugaaaaaaaaaaaaaaaaaaaaa

SEQ ID NO: 367 - DNA, 138 bp, Artificial Sequence
  E190
gggagccaccauggacuacaaggacgacgacgacaagaucaucgacuauaaagacgacgacgauaaagguggcgacuauaaggacgacgacgacaaacaccaccaccaccaccactgaaaaaaaaaaaaaaaaaaaaa

SEQ ID NO: 368 - RNA, 53 nt, Artificial Sequence
  E190-1
gggagccaccauggacuacaaggacgacgacgacaagaucaucgacuauaaag

SEQ ID NO: 369 - DNA, 85 bp, Artificial Sequence; identical to SEQ ID NO: 7
  E190-2

SEQ ID NO: 370 - DNA, 138 bp, Artificial Sequence; identical to SEQ ID NO: 367
  E191

SEQ ID NO: 371 - RNA, 53 nt, Artificial Sequence; identical to SEQ ID NO: 368
  E191-1

SEQ ID NO: 372 - DNA, 85 bp, Artificial Sequence; identical to SEQ ID NO: 7
  E191-2

SEQ ID NO: 373 - RNA, 185 nt, Artificial Sequence
  E192
gggagaauacaagcuacuuguucuuuuugcagccaccauggacuacaaggacgacgacgacaagaucaucgacuauaaagacgacgacgauaaagguggcgacuauaaggacgacgacgacaaacaccaccaccaccaccacugaaaaaaaaaaaaaaaaaaaaaaaaaaaaaaaaaaaaaaaaa

SEQ ID NO: 374 - DNA, 165 bp, Artificial Sequence; identical to SEQ ID NO: 5
  E193

SEQ ID NO: 375 - RNA, 80 nt, Artificial Sequence; identical to SEQ ID NO: 2
  E193-1

SEQ ID NO: 376 - DNA, 85 bp, Artificial Sequence; identical to SEQ ID NO: 7
  E193-2

SEQ ID NO: 377 - DNA, 165 bp, Artificial Sequence
  E194
  misc_feature (8)..(8): rSpacer
  misc_feature (11)..(11): rSpacer
  misc_feature (14)..(14): rSpacer
  misc_feature (17)..(17): rSpacer
  misc_feature (20)..(20): rSpacer
  misc_feature (23)..(23): rSpacer
  misc_feature (26)..(26): rSpacer
gggagaanacnagnuanuunuunuunuugcagccaccauggacuacaaggacgacgacgacaagaucaucgacuauaaagacgacgacgauaaagguggcgacuauaaggacgacgacgacaaacaccaccaccaccaccactgaaaaaaaaaaaaaaaaaaaaa

SEQ ID NO: 378 - RNA, 80 nt, Artificial Sequence
  E194-1
  misc_feature (8)..(8): rSpacer
  misc_feature (11)..(11): rSpacer
  misc_feature (14)..(14): rSpacer
  misc_feature (17)..(17): rSpacer
  misc_feature (20)..(20): rSpacer
  misc_feature (23)..(23): rSpacer
  misc_feature (26)..(26): rSpacer
gggagaanacnagnuanuunuunuunuugcagccaccauggacuacaaggacgacgacgacaagaucaucgacuauaaag

SEQ ID NO: 379 - DNA, 85 bp, Artificial Sequence; identical to SEQ ID NO: 7
  E194-2

SEQ ID NO: 380 - DNA, 165 bp, Artificial Sequence
  E195
  misc_feature (32)..(32): rSpacer
  misc_feature (35)..(35): rSpacer
gggagaauacaagcuacuuguucuuuuugcanccnccauggacuacaaggacgacgacgacaagaucaucgacuauaaagacgacgacgauaaagguggcgacuauaaggacgacgacgacaaacaccaccaccaccaccactgaaaaaaaaaaaaaaaaaaaaa

SEQ ID NO: 381 - RNA, 80 nt, Artificial Sequence
  E195-1
  misc_feature (32)..(32): rSpacer
  misc_feature (35)..(35): rSpacer
gggagaauacaagcuacuuguucuuuuugcanccnccauggacuacaaggacgacgacgacaagaucaucgacuauaaag

SEQ ID NO: 382 - DNA, 85 bp, Artificial Sequence; identical to SEQ ID NO: 7
  E195-2

SEQ ID NO: 383 - DNA, 165 bp, Artificial Sequence
  E196
  misc_feature (38)..(38): rSpacer
  misc_feature (41)..(41): rSpacer
gggagaauacaagcuacuuguucuuuuugcagccaccnugnacuacaaggacgacgacgacaagaucaucgacuauaaagacgacgacgauaaagguggcgacuauaaggacgacgacgacaaacaccaccaccaccaccactgaaaaaaaaaaaaaaaaaaaaa

SEQ ID NO: 384 - RNA, 80 nt, Artificial Sequence
  E196-1
  misc_feature (38)..(38): rSpacer
  misc_feature (41)..(41): rSpacer
gggagaauacaagcuacuuguucuuuuugcagccaccnugnacuacaaggacgacgacgacaagaucaucgacuauaaag

SEQ ID NO: 385 - DNA, 85 bp, Artificial Sequence; identical to SEQ ID NO: 7
  E196-2

SEQ ID NO: 386 - DNA, 165 bp, Artificial Sequence
  E197
  misc_feature (110)..(110): rSpacer
  misc_feature (113)..(113): rSpacer
gggagaauacaagcuacuuguucuuuuugcagccaccauggacuacaaggacgacgacgacaagaucaucgacuauaaagacgacgacgauaaagguggcgacuauaagnacnacgacgacaaacaccaccaccaccaccactgaaaaaaaaaaaaaaaaaaaaa

SEQ ID NO: 387 - RNA, 80 nt, Artificial Sequence; identical to SEQ ID NO: 2
  E197-1

SEQ ID NO: 388 - DNA, 85 bp, Artificial Sequence
  E197-2
  misc_feature (30)..(30): rSpacer
  misc_feature (33)..(33): rSpacer
acgacgacgauaaagguggcgacuauaagnacnacgacgacaaacaccaccaccaccaccactgaaaaaaaaaaaaaaaaaaaaa

SEQ ID NO: 389 - DNA, 165 bp, Artificial Sequence
  E198
  misc_feature (158)..(158): rSpacer
  misc_feature (161)..(161): rSpacer
gggagaauacaagcuacuuguucuuuuugcagccaccauggacuacaaggacgacgacgacaagaucaucgacuauaaagacgacgacgauaaagguggcgacuauaaggacgacgacgacaaacaccaccaccaccaccactgaaaaaaaaaaaaanaanaaaa

SEQ ID NO: 390 - RNA, 80 nt, Artificial Sequence; identical to SEQ ID NO: 2
  E198-1

SEQ ID NO: 391 - DNA, 85 bp, Artificial Sequence
  E198-2
  misc_feature (78)..(78): rSpacer
  misc_feature (81)..(81): rSpacer
acgacgacgauaaagguggcgacuauaaggacgacgacgacaaacaccaccaccaccaccactgaaaaaaaaaaaaanaanaaaa

SEQ ID NO: 392 - DNA, 165 bp, Artificial Sequence
  E199
  misc_feature (146)..(146): rSpacer
  misc_feature (149)..(149): rSpacer
  misc_feature (152)..(152): rSpacer
  misc_feature (155)..(155): rSpacer
  misc_feature (158)..(158): rSpacer
  misc_feature (161)..(161): rSpacer
gggagaauacaagcuacuuguucuuuuugcagccaccauggacuacaaggacgacgacgacaagaucaucgacuauaaagacgacgacgauaaagguggcgacuauaaggacgacgacgacaaacaccaccaccaccaccactganaanaanaanaanaanaaaa

SEQ ID NO: 393 - RNA, 80 nt, Artificial Sequence; identical to SEQ ID NO: 2
  E199-1

SEQ ID NO: 394 - DNA, 85 bp, Artificial Sequence
  E199-2
  misc_feature (66)..(66): rSpacer
  misc_feature (69)..(69): rSpacer
  misc_feature (72)..(72): rSpacer
  misc_feature (75)..(75): rSpacer
  misc_feature (78)..(78): rSpacer
  misc_feature (81)..(81): rSpacer
acgacgacgauaaagguggcgacuauaaggacgacgacgacaaacaccaccaccaccaccactganaanaanaanaanaanaaaa

SEQ ID NO: 395 - DNA, 91 bp, Artificial Sequence
  E200
  misc_feature (19)..(19): C2
gggagaauacaagcuacunguucuuuuugcagccaccauggacuauaaggacgacgacgacaaagguggccaccaccaccaccaccactga

SEQ ID NO: 396 - DNA, 91 bp, Artificial Sequence
  E201
  misc_feature (19)..(19): C2
  misc_feature (23)..(23): C2
gggagaauacaagcuacunguunuuuuugcagccaccauggacuauaaggacgacgacgacaaagguggccaccaccaccaccaccactga

SEQ ID NO: 397 - DNA, 90 bp, Artificial Sequence
  E202
  misc_feature (19)..(19): Spacer9
gggagaauacaagcuacunuucuuuuugcagccaccauggacuauaaggacgacgacgacaaagguggccaccaccaccaccaccactga

SEQ ID NO: 398 - DNA, 90 bp, Artificial Sequence
  E203
  misc_feature (23)..(23): Spacer9
gggagaauacaagcuacuuguunuuuugcagccaccauggacuauaaggacgacgacgacaaagguggccaccaccaccaccaccactga

SEQ ID NO: 399 - DNA, 91 bp, Artificial Sequence; identical to SEQ ID NO: 198
  E204

SEQ ID NO: 400 - DNA, 91 bp, Artificial Sequence; identical to SEQ ID NO: 198
  E205

SEQ ID NO: 401 - DNA, 91 bp, Artificial Sequence; identical to SEQ ID NO: 198
  E206

SEQ ID NO: 402 - RNA, 91 nt, Artificial Sequence; identical to SEQ ID NO: 89
  E207

SEQ ID NO: 403 - RNA, 91 nt, Artificial Sequence; identical to SEQ ID NO: 89
  E208

SEQ ID NO: 404 - DNA, 91 bp, Artificial Sequence; identical to SEQ ID NO: 198
  E209

SEQ ID NO: 405 - DNA, 91 bp, Artificial Sequence; identical to SEQ ID NO: 198
  E210

SEQ ID NO: 406 - DNA, 91 bp, Artificial Sequence; identical to SEQ ID NO: 198
  E211

SEQ ID NO: 407 - RNA, 91 nt, Artificial Sequence; identical to SEQ ID NO: 89
  E212

SEQ ID NO: 408 - RNA, 91 nt, Artificial Sequence; identical to SEQ ID NO: 89
  E213

SEQ ID NO: 409 - DNA, 95 bp, Artificial Sequence
  E214
gggggagaauacaagcuacuuguucuuuuugcagccaccauggacuauaaggacgacgacgacaaagguggccaccaccaccaccaccactgaaa

SEQ ID NO: 410 - DNA, 165 bp, Artificial Sequence
  E215
gggagaatacaagcuacuuguucuutuugcagccaccauggacuacaaggacgacgacgacaagaucaucgacuauaaagacgacgacgauaaagguggcgacuauaaggacgacgacgacaaacaccaccaccaccaccactgaaaaaaaaaaaaaaaaaaaaa

SEQ ID NO: 411 - DNA, 80 bp, Artificial Sequence
  E215-1
gggagaatacaagcuacuuguucuutuugcagccaccauggacuacaaggacgacgacgacaagaucaucgacuauaaag

SEQ ID NO: 412 - DNA, 85 bp, Artificial Sequence; identical to SEQ ID NO: 7
  E215-2

SEQ ID NO: 413 - DNA, 165 bp, Artificial Sequence
  E216
gggagaatacaagcuacutgutcuttutgcagccaccauggacuacaaggacgacgacgacaagaucaucgacuauaaagacgacgacgauaaagguggcgacuauaaggacgacgacgacaaacaccaccaccaccaccactgaaaaaaaaaaaaaaaaaaaaa

SEQ ID NO: 414 - DNA, 80 bp, Artificial Sequence
  E216-1
gggagaatacaagcuacutgutcuttutgcagccaccauggacuacaaggacgacgacgacaagaucaucgacuauaaag

SEQ ID NO: 415 - DNA, 85 bp, Artificial Sequence; identical to SEQ ID NO: 7
  E216-2

SEQ ID NO: 416 - RNA, 194 nt, Artificial Sequence
  E217
cauaaacccuggcgcgcucgcgggccggcacucuucugguccccacagacucagagagaacccaccauggacuacaaggacgacgacgacaagaucaucgacuauaaagacgacgacgauaaagguggcgacuauaaggacgacgacgacaaacaccaccaccaccaccacugaaaaaaaaaaaaaaaaaaaaa

SEQ ID NO: 417 - RNA, 81 nt, Artificial Sequence
  E217-1
cauaaacccuggcgcgcucgcgggccggcacucuucugguccccacagacucagagagaacccaccauggacuacaaggac

SEQ ID NO: 418 - RNA, 57 nt, Artificial Sequence
  E217-2
gacgacgacaagaucaucgacuauaaagacgacgacgauaaagguggcgacuauaag

SEQ ID NO: 419 - RNA, 56 nt, Artificial Sequence
  E217-3
gacgacgacgacaaacaccaccaccaccaccacugaaaaaaaaaaaaaaaaaaaaa

SEQ ID NO: 420 - DNA, 30 bp, Artificial Sequence
  template DNA 2
gatcttgtcgtcgtcgtccttgtagtccat

SEQ ID NO: 421 - DNA, 30 bp, Artificial Sequence
  template DNA 3
tttgtcgtcgtcgtccttatagtcgccacc

SEQ ID NO: 422 - DNA, 194 bp, Artificial Sequence
  E218
cataaacccuggcgcgcucgcgggccggcacucuucugguccccacagacucagagagaacccaccauggacuacaaggacgacgacgacaagaucaucgacuauaaagacgacgacgauaaagguggcgacuauaaggacgacgacgacaaacaccaccaccaccaccactgaaaaaaaaaaaaaaaaaaaaa

SEQ ID NO: 423 - DNA, 81 bp, Artificial Sequence
  E218-1
cataaacccuggcgcgcucgcgggccggcacucuucugguccccacagacucagagagaacccaccauggacuacaaggac

SEQ ID NO: 424 - RNA, 57 nt, Artificial Sequence; identical to SEQ ID NO: 418
  E218-2

SEQ ID NO: 425 - DNA, 56 bp, Artificial Sequence
  E218-3
gacgacgacgacaaacaccaccaccaccaccactgaaaaaaaaaaaaaaaaaaaaa

SEQ ID NO: 426 - DNA, 194 bp, Artificial Sequence; identical to SEQ ID NO: 422
  E219

SEQ ID NO: 427 - DNA, 81 bp, Artificial Sequence; identical to SEQ ID NO: 423
  E219-1

SEQ ID NO: 428 - RNA, 57 nt, Artificial Sequence; identical to SEQ ID NO: 418
  E219-2

SEQ ID NO: 429 - DNA, 56 bp, Artificial Sequence; identical to SEQ ID NO: 425
  E219-3

SEQ ID NO: 430 - protein, 35 aa, Artificial Sequence
  translated product standard
MDYKDDDDKIIDYKDDDDKGGDYKDDDDKHHHHHH

SEQ ID NO: 431 - DNA, 25 bp, Artificial Sequence
  RT primer
tcagtggtggtggtggtggtgtttg

SEQ ID NO: 432 - DNA, 20 bp, Artificial Sequence
  Fw primer
atcttgtcgtcgtcgtcctt

SEQ ID NO: 433 - DNA, 23 bp, Artificial Sequence
  Rv primer
gaatacaagctacttgttctttt

SEQ ID NO: 434 - DNA, 11 bp, Artificial Sequence
  Taqman MGB Probe
cagccaccatg

SEQ ID NO: 435 - protein, 17 aa, Artificial Sequence
  translated product standard
MDYKDDDDKGGHHHHHH

SEQ ID NO: 436 - RNA, 66 nt, Artificial Sequence
  N1
gggaaauaagagagaaaagaagaguaagaagaaauauaagagccaccaugaacuuucugcugucuu

SEQ ID NO: 437 - RNA, 66 nt, Artificial Sequence; identical to SEQ ID NO: 436
  N2

SEQ ID NO: 438 - RNA, 66 nt, Artificial Sequence
  N3
  misc_feature (8)..(9): Am6(F)
  misc_feature (11)..(11): Am6(F)
  misc_feature (13)..(13): Am6(F)
  misc_feature (15)..(18): Am6(F)
  misc_feature (20)..(21): Am6(F)
  misc_feature (23)..(23): Am6(F)
  misc_feature (26)..(27): Am6(F)
  misc_feature (29)..(30): Am6(F)
  misc_feature (32)..(34): Am6(F)
  misc_feature (36)..(36): Am6(F)
  misc_feature (38)..(39): Am6(F)
  misc_feature (41)..(41): Am6(F)
  misc_feature (45)..(45): Am6(F)
gggaaaunngngngnnnngnngngunngnngnnnununngngccnccaugaacuuucugcugucuu

SEQ ID NO: 439 - DNA, 802 bp, Artificial Sequence
  GN
aattcagtacttaatacgactcactatagggtgcattggagccttgccttgctgctctacctccaccatgccaagtggtcccaggctgcacccatggcagaaggaggagggcagaatcatcacgaagtggtgaagttcatggatgtctatcagcgcagctactgccatccaatcgagaccctggtggacatcttccaggagtaccctgatgagatcgagtacatcttcaagccatcctgtgtgcccctgatgcgatgcgggggctgctgcaatgacgagggcctggagtgtgtgcccactgaggagtccaacatcaccatgcagattatgcggatcaaacctcaccaaggccagcacataggagagatgagcttcctacagcacaacaaatgtgaatgcagaccaaagaaagatagagcaagacaagaaaatccctgtgggccttgctcagagcggagaaagcatttgtttgtacaagatccgcagacgtgtaaatgttcctgcaaaaacacagactcgcgttgcaaggcgaggcagcttgagttaaacgaacgtacttgcagatgtgacaagccgaggcggtgataataggctggagcctcggtggccatgcttcttgccccttgggcctccccccagcccctcctccccttcctgcacccgtacccccgtggtctttgaataaagtctgagtgggcggcaaaaaaaaaaaaaaaaaaaaaaaaaaaaaaaaaaaaaaaaaaaaaaaaaaaaaaaaaaaaaaaaaaaaaaaaaaaaaaaaaaaaaaaaaaaaaaaaaaaat

SEQ ID NO: 440 - DNA, 30 bp, Artificial Sequence
  template DNA 4
ggctccaatgcacccaagacagcagaaagt

SEQ ID NO: 441 - RNA, 844 nt, Artificial Sequence
  VEGF-1
gggaaauaagagagaaaagaagaguaagaagaaauauaagagccaccaugaacuuucugcugucuugggugcauuggagccuugccuugcugcucuaccuccaccaugccaaguggucccaggcugcacccauggcagaaggaggagggcagaaucaucacgaaguggugaaguucauggaugucuaucagcgcagcuacugccauccaaucgagacccugguggacaucuuccaggaguacccugaugagaucgaguacaucuucaagccauccugugugccccugaugcgaugcgggggcugcugcaaugacgagggccuggagugugugcccacugaggaguccaacaucaccaugcagauuaugcggaucaaaccucaccaaggccagcacauaggagagaugagcuuccuacagcacaacaaaugugaaugcagaccaaagaaagauagagcaagacaagaaaaucccugugggccuugcucagagcggagaaagcauuuguuuguacaagauccgcagacguguaaauguuccugcaaaaacacagacucgcguugcaaggcgaggcagcuugaguuaaacgaacguacuugcagaugugacaagccgaggcggugauaauaggcuggagccucgguggccaugcuucuugccccuugggccuccccccagccccuccuccccuuccugcacccguacccccguggucuuugaauaaagucugagugggcggcaaaaaaaaaaaaaaaaaaaaaaaaaaaaaaaaaaaaaaaaaaaaaaaaaaaaaaaaaaaaaaaaaaaaaaaaaaaaaaaaaaaaaaaaaaaaaaaaaaaaucuag

SEQ ID NO: 442 - RNA, 844 nt, Artificial Sequence
  VEGF-2
  misc_feature (8)..(8): Am6(M)
  misc_feature (9)..(9): Am6(F)
  misc_feature (11)..(11): Am6(F)
  misc_feature (13)..(13): Am6(F)
  misc_feature (15)..(15): Am6(F)
  misc_feature (16)..(16): Am6(M)
  misc_feature (17)..(17): Am6(F)
  misc_feature (18)..(18): Am6(M)
  misc_feature (20)..(20): Am6(M)
  misc_feature (21)..(21): Am6(F)
  misc_feature (23)..(23): Am6(F)
  misc_feature (26)..(26): Am6(M)
  misc_feature (27)..(27): Am6(F)
  misc_feature (29)..(29): Am6(M)
  misc_feature (30)..(30): Am6(F)
  misc_feature (32)..(32): Am6(M)
  misc_feature (33)..(33): Am6(F)
  misc_feature (34)..(34): Am6(M)
  misc_feature (36)..(36): Am6(M)
  misc_feature (38)..(38): Am6(M)
  misc_feature (39)..(39): Am6(F)
  misc_feature (41)..(41): Am6(F)
  misc_feature (45)..(45): Am6(F)
gggaaaunngngngnnnngnngngunngnngnnnununngngccnccaugaacuuucugcugucuugggugcauuggagccuugccuugcugcucuaccuccaccaugccaaguggucccaggcugcacccauggcagaaggaggagggcagaaucaucacgaaguggugaaguucauggaugucuaucagcgcagcuacugccauccaaucgagacccugguggacaucuuccaggaguacccugaugagaucgaguacaucuucaagccauccugugugccccugaugcgaugcgggggcugcugcaaugacgagggccuggagugugugcccacugaggaguccaacaucaccaugcagauuaugcggaucaaaccucaccaaggccagcacauaggagagaugagcuuccuacagcacaacaaaugugaaugcagaccaaagaaagauagagcaagacaagaaaaucccugugggccuugcucagagcggagaaagcauuuguuuguacaagauccgcagacguguaaauguuccugcaaaaacacagacucgcguugcaaggcgaggcagcuugaguuaaacgaacguacuugcagaugugacaagccgaggcggugauaauaggcuggagccucgguggccaugcuucuugccccuugggccuccccccagccccuccuccccuuccugcacccguacccccguggucuuugaauaaagucugagugggcggcaaaaaaaaaaaaaaaaaaaaaaaaaaaaaaaaaaaaaaaaaaaaaaaaaaaaaaaaaaaaaaaaaaaaaaaaaaaaaaaaaaaaaaaaaaaaaaaaaaaaucuag

SEQ ID NO: 443 - RNA, 844 nt, Artificial Sequence; identical to SEQ ID NO: 441
  VEGF-3

SEQ ID NO: 444 - DNA, 635 bp, Artificial Sequence
  GO
gatccgaaattaatacgactcactatagatggactacaaggacgacgacgacaagatcatcgactataaagacgacgacgataaaggtggcgactataaggacgacgacgacaaacaccaccaccaccaccacgctgcaatcagtctgattgcggcgttagcggtagatcgcgttatcggcatggaaaacgccatgccgtggaacctgcctgccgatctcgcctggtttaaacgcaacaccttaaataaacccgtgattatgggccgccatacctgggaatcaatcggtcgtccgttgccaggacgcaaaaatattatcctcagcagtcaaccgggtacggacgatcgcgtaacgtgggtgaagtcggtggatgaagccatcgcggcgtgtggtgacgtaccagaaatcatggtgattggcggcggtcgcgtttatgaacagttcttgccaaaagcgcaaaaactgtatctgacgcatatcgacgcagaagtggaaggcgacacccatttcccggattacgagccggatgactgggaatcggtattcagcgaattccacgatgctgatgcgcagaactctcacagctattgctttgagattctggagcggcggtaatgaataactaatccctgca

SEQ ID NO: 445 - DNA, 90 bp, Artificial Sequence
  primer P1
ttggaccctcgtacagaagctaatacgactcactatagggagaatacaagctacttgttctttttgcagccaccatggactacaaggacg

SEQ ID NO: 446 - DNA, 45 bp, Artificial Sequence
  primer P2
tttttttttttttttttttttcagtggtggtggtggtggtgtttg

SEQ ID NO: 447 - RNA, 166 nt, Artificial Sequence
  IVT-1
ggggagaauacaagcuacuuguucuuuuugcagccaccauggacuacaaggacgacgacgacaagaucaucgacuauaaagacgacgacgauaaagguggcgacuauaaggacgacgacgacaaacaccaccaccaccaccacugaaaaaaaaaaaaaaaaaaaaa

SEQ ID NO: 448 - RNA, 150 nt, Artificial Sequence
  E220
gggagaauacaagcuacuuguucuuuuugcagccaccauggacuacaaggacgacgacgacaagaucaucgacuauaaagacgacgacgauaaagguggcgacuauaaggacgacgacgacaaacaccaccaccaccaccacugaaaaaa

SEQ ID NO: 449 - RNA, 80 nt, Artificial Sequence; identical to SEQ ID NO: 2
  E220-1

SEQ ID NO: 450 - RNA, 70 nt, Artificial Sequence
  E220-2
acgacgacgauaaagguggcgacuauaaggacgacgacgacaaacaccaccaccaccaccacugaaaaaa

SEQ ID NO: 451 - RNA, 155 nt, Artificial Sequence
  E221
gggagaauacaagcuacuuguucuuuuugcagccaccauggacuacaaggacgacgacgacaagaucaucgacuauaaagacgacgacgauaaagguggcgacuauaaggacgacgacgacaaacaccaccaccaccaccacugaaaaaaaaaaa

SEQ ID NO: 452 - RNA, 80 nt, Artificial Sequence; identical to SEQ ID NO: 2
  E221-1

SEQ ID NO: 453 - RNA, 75 nt, Artificial Sequence
  E221-2
acgacgacgauaaagguggcgacuauaaggacgacgacgacaaacaccaccaccaccaccacugaaaaaaaaaaa

SEQ ID NO: 454 - DNA, 150 bp, Artificial Sequence
  E222
gggagaauacaagcuacuuguucuuuuugcagccaccauggacuacaaggacgacgacgacaagaucaucgacuauaaagacgacgacgauaaagguggcgacuauaaggacgacgacgacaaacaccaccaccaccaccactgaaaaaa

SEQ ID NO: 455 - RNA, 80 nt, Artificial Sequence; identical to SEQ ID NO: 2
  E222-1

SEQ ID NO: 456 - DNA, 70 bp, Artificial Sequence
  E222-2
acgacgacgauaaagguggcgacuauaaggacgacgacgacaaacaccaccaccaccaccactgaaaaaa

SEQ ID NO: 457 - DNA, 155 bp, Artificial Sequence
  E223
gggagaauacaagcuacuuguucuuuuugcagccaccauggacuacaaggacgacgacgacaagaucaucgacuauaaagacgacgacgauaaagguggcgacuauaaggacgacgacgacaaacaccaccaccaccaccactgaaaaaaaaaaa

SEQ ID NO: 458 - RNA, 80 nt, Artificial Sequence; identical to SEQ ID NO: 2
  E223-1

SEQ ID NO: 459 - DNA, 75 bp, Artificial Sequence
  E223-2
acgacgacgauaaagguggcgacuauaaggacgacgacgacaaacaccaccaccaccaccactgaaaaaaaaaaa

SEQ ID NO: 460 - DNA, 165 bp, Artificial Sequence; identical to SEQ ID NO: 5
  E224

SEQ ID NO: 461 - RNA, 80 nt, Artificial Sequence; identical to SEQ ID NO: 2
  E224-1

SEQ ID NO: 462 - DNA, 85 bp, Artificial Sequence; identical to SEQ ID NO: 7
  E224-2

SEQ ID NO: 463 - DNA, 165 bp, Artificial Sequence; identical to SEQ ID NO: 5
  E225

SEQ ID NO: 464 - RNA, 80 nt, Artificial Sequence; identical to SEQ ID NO: 2
  E225-1

SEQ ID NO: 465 - DNA, 85 bp, Artificial Sequence; identical to SEQ ID NO: 7
  E225-2

SEQ ID NO: 466 - RNA, 67 nt, Artificial Sequence
  E226
gggagccaccauggacuauaaggacgacgacgacaaagguggcagccaccaccaccaccaccacuga

SEQ ID NO: 467 - DNA, 67 bp, Artificial Sequence
  E227
gggagccaccauggacuauaaggacgacgacgacaaagguggcagccaccaccaccaccaccactga

SEQ ID NO: 468 - DNA, 67 bp, Artificial Sequence; identical to SEQ ID NO: 467
  E228

SEQ ID NO: 469 - DNA, 67 bp, Artificial Sequence; identical to SEQ ID NO: 467
  E229

SEQ ID NO: 470 - RNA, 91 nt, Artificial Sequence; identical to SEQ ID NO: 89
  E230

SEQ ID NO: 471 - RNA, 91 nt, Artificial Sequence; identical to SEQ ID NO: 89
  E231

SEQ ID NO: 472 - RNA, 91 nt, Artificial Sequence; identical to SEQ ID NO: 89
  E232

SEQ ID NO: 473 - RNA, 91 nt, Artificial Sequence; identical to SEQ ID NO: 89
  E233

SEQ ID NO: 474 - DNA, 91 bp, Artificial Sequence
  E234
gggagaauacaagcuacuuguucuuuuugcagccaccauggactauaaggacgacgacgacaaagguggccaccaccaccaccaccacuga

SEQ ID NO: 475 - DNA, 91 bp, Artificial Sequence; identical to SEQ ID NO: 198
  E235

SEQ ID NO: 476 - RNA, 91 nt, Artificial Sequence; identical to SEQ ID NO: 89
  E236

SEQ ID NO: 477 - DNA, 91 bp, Artificial Sequence; identical to SEQ ID NO: 198
  E237

SEQ ID NO: 478 - RNA, 91 nt, Artificial Sequence; identical to SEQ ID NO: 89
  E238

SEQ ID NO: 479 - DNA, 91 bp, Artificial Sequence; identical to SEQ ID NO: 198
  E239

SEQ ID NO: 480 - DNA, 91 bp, Artificial Sequence; identical to SEQ ID NO: 198
  E240